European Patent Application EP 4 414 386 A1, published August 14, 2024. Title: METHOD OF CHEMICAL SYNTHESIS OF SINGLE-CHAIN ANTIBODY FRAGMENTS AND PRODUCTS THEREBY OBTAINED. Applicant: FIGINI Mariangela. The sequence listing filed with the application follows.

SEQUENCE LISTING (1 sequence)

SEQ ID NO: 1 - protein, 254 aa, unidentified
EVKLQESGPGLVKPSQSLSLTCSVTGYSITSGYYWNWIRQFPGNKLEWMGSISFDGNNNYNPSLRNRISITRDTSKNQFFLKLNSVTTEDTATYYCAREGDYYGSSFFTYWGQGTLVTVSSGGGGSGGGGSGGGGSALDIVMTQSPASLSASVGETVTLTCGASENIYGALNWYQRKQGKSPQLLIYGATNLADGMSSRFSGSGSGRQYSLKISSLHPDDVATYYCQNVFRTYTFGGGTKLEIKRAAAHHHHHH